European Patent Specification EP 3 598 104 B1, published March 29, 2023. Title: ANALYSIS DEVICE, ANALYSIS KIT AND ANALYSIS SYSTEM. Applicant: TOPPAN PRINTING CO., LTD. The sequence listing filed with the application follows.

SEQUENCE LISTING (7 sequences)

SEQ ID NO: 1 - DNA, 56 bp, Homo sapiens
ccgaagggcatgagctgcgtgatgagctgcacggtggaggtgaggcagatgcccag

SEQ ID NO: 2 - DNA, 56 bp, Homo sapiens
ccgaagggcatgagctgcatgatgagctgcacggtggaggtgaggcagatgcccag

SEQ ID NO: 3 - DNA, 24 bp, Artificial Sequence
  Synthesized oligonucleotide
cgcgccgaggcgcagctcatgccc

SEQ ID NO: 4 - DNA, 26 bp, Artificial Sequence
  Synthesized oligonucleotide
acggacgcggagtgcagctcatgccc

SEQ ID NO: 5 - DNA, 19 bp, Artificial Sequence
  Synthesized oligonucleotide
ccaccgtgcarctcatcaa

SEQ ID NO: 6 - DNA, 10 bp, Artificial Sequence
  Synthesized oligonucleotide
cgcgccgagg

SEQ ID NO: 7 - DNA, 12 bp, Artificial Sequence
  Synthesized oligonucleotide
acggacgcggag